European Patent Specification EP 4 085 256 B1, published January 24, 2024. Title: TEST AND IN VITRO DIAGNOSIS OF IRRITABLE BOWEL SYNDROME. Applicant: IMMUNDIAGNOSTIK AG. Application DE102020101864.9. The sequence listing filed with the application follows.

SEQUENCE LISTING (1 sequence)

SEQ ID NO: 1 - protein, 15 aa, Homo sapiens
CRRDYPGPGGSILQP